European Patent Specification EP 3 897 672 B1, published August 9, 2023. Title: COMBINATION HBV THERAPY. Applicant: Humabs BioMed SA Vir Biotechnology, Inc. Bakardjiev, Anna Pang, Phillip S. Corti, Davide. Application PCT. The sequence listing filed with the application follows.

SEQUENCE LISTING (109 sequences)

SEQ ID NO: 1 - DNA, 3182 bp, Hepatitis B Virus
  Hepatitis B Virus genome, NC_003977.2
aattccacaaccttccaccaaactctgcaagatcccagagtgagaggcctgtatttccctgctggtggctccagttcaggaacagtaaaccctgttctgactactgcctctcccttatcgtcaatcttctcgaggattggggaccctgcgctgaacatggagaacatcacatcaggattcctaggaccccttctcgtgttacaggcggggtttttcttgttgacaagaatcctcacaataccgcagagtctagactcgtggtggacttctctcaattttctagggggaactaccgtgtgtcttggccaaaattcgcagtccccaacctccaatcactcaccaacctcttgtcctccaacttgtcctggttatcgctggatgtgtctgcggcgttttatcatcttcctcttcatcctgctgctatgcctcatcttcttgttggttcttctggactatcaaggtatgttgcccgtttgtcctctaattccaggatcctcaacaaccagcacgggaccatgccggacctgcatgactactgctcaaggaacctctatgtatccctcctgttgctgtaccaaaccttcggacggaaattgcacctgtattcccatcccatcatcctgggctttcggaaaattcctatgggagtgggcctcagcccgtttctcctggctcagtttactagtgccatttgttcagtggttcgtagggctttcccccactgtttggctttcagttatatggatgatgtggtattgggggccaagtctgtacagcatcttgagtccctttttaccgctgttaccaattttcttttgtctttgggtatacatttaaaccctaacaaaacaaagagatggggttactctctaaattttatgggttatgtcattggatgttatgggtccttgccacaagaacacatcatacaaaaaatcaaagaatgttttagaaaacttcctattaacaggcctattgattggaaagtatgtcaacgaattgtgggtcttttgggttttgctgccccttttacacaatgtggttatcctgcgttgatgcctttgtatgcatgtattcaatctaagcaggctttcactttctcgccaacttacaaggcctttctgtgtaaacaatacctgaacctttaccccgttgcccggcaacggccaggtctgtgccaagtgtttgctgacgcaacccccactggctggggcttggtcatgggccatcagcgcatgcgtggaaccttttcggctcctctgccgatccatactgcggaactcctagccgcttgttttgctcgcagcaggtctggagcaaacattatcgggactgataactctgttgtcctatcccgcaaatatacatcgtttccatggctgctaggctgtgctgccaactggatcctgcgcgggacgtcctttgtttacgtcccgtcggcgctgaatcctgcggacgacccttctcggggtcgcttgggactctctcgtccccttctccgtctgccgttccgaccgaccacggggcgcacctctctttacgcggactccccgtctgtgccttctcatctgccggaccgtgtgcacttcgcttcacctctgcacgtcgcatggagaccaccgtgaacgcccaccaaatattgcccaaggtcttacataagaggactcttggactctcagcaatgtcaacgaccgaccttgaggcatacttcaaagactgtttgtttaaagactgggaggagttgggggaggagattaggttaaaggtctttgtactaggaggctgtaggcataaattggtctgcgcaccagcaccatgcaactttttcacctctgcctaatcatctcttgttcatgtcctactgttcaagcctccaagctgtgccttgggtggctttggggcatggacatcgacccttataaagaatttggagctactgtggagttactctcgtttttgccttctgacttctttccttcagtacgagatcttctagataccgcctcagctctgtatcgggaagccttagagtctcctgagcattgttcacctcaccatactgcactcaggcaagcaattctttgctggggggaactaatgactctagctacctgggtgggtgttaatttggaagatccagcgtctagagacctagtagtcagttatgtcaacactaatatgggcctaaagttcaggcaactcttgtggtttcacatttcttgtctcacttttggaagagaaacagttatagagtatttggtgtctttcggagtgtggattcgcactcctccagcttatagaccaccaaatgcccctatcctatcaacacttccggagactactgttgttagacgacgaggcaggtcccctagaagaagaactccctcgcctcgcagacgaaggtctcaatcgccgcgtcgcagaagatctcaatctcgggaatctcaatgttagtattccttggactcataaggtggggaactttactgggctttattcttctactgtacctgtctttaatcctcattggaaaacaccatcttttcctaatatacatttacaccaagacattatcaaaaaatgtgaacagtttgtaggcccactcacagttaatgagaaaagaagattgcaattgattatgcctgccaggttttatccaaaggttaccaaatatttaccattggataagggtattaaaccttattatccagaacatctagttaatcattacttccaaactagacactatttacacactctatggaaggcgggtatattatataagagagaaacaacacatagcgcctcattttgtgggtcaccatattcttgggaacaagatctacagcatggggcagaatctttccaccagcaatcctctgggattctttcccgaccaccagttggatccagccttcagagcaaacaccgcaaatccagattgggacttcaatcccaacaaggacacctggccagacgccaacaaggtaggagctggagcattcgggctgggtttcaccccaccgcacggaggccttttggggtggagccctcaggctcagggcatactacaaactttgccagcaaatccgcctcctgcctccaccaatcgccagtcaggaaggcagcctaccccgctgtctccacctttgagaaacactcatcctcaggccatgcagtgg

SEQ ID NO: 2 - DNA, 18 bp, Hepatitis B Virus
  Hepatitis B Virus genome, nucleotides 1579-1597 of NC_003977.2
gtgtgcacttcgcttcac

SEQ ID NO: 3 - RNA, 19 nt, Artificial Sequence
  Synthetic sequence HBV02, sense strand
gugugcacuucgcuucaca

SEQ ID NO: 4 - RNA, 21 nt, Artificial Sequence
  Synthetic sequence HBV02, antisense strand
ugugaagcgaagugcacacuu

SEQ ID NO: 5 - RNA, 19 nt, Artificial Sequence
  Synthetic oligonucleotide (HBV01, sense strand)
gugugcacuucgcuucaca

SEQ ID NO: 6 - RNA, 21 nt, Artificial Sequence
  Synthetic oligonucleotide (HBV01, antisense strand)
ugugaagcgaagugcacacuu

SEQ ID NO: 7 - RNA, 19 nt, Artificial Sequence
  Synthetic oligonucleotide (HBV02, sense strand)
gugugcacuucgcuucaca

SEQ ID NO: 8 - RNA, 21 nt, Artificial Sequence
  Synthetic oligonucleotide (HBV02, antisense strand)
ugugaagcgaagugcacacuu

SEQ ID NO: 9 - protein, 16 aa, Artificial Sequence
  Membrane translocation sequence-containing peptide RFGF
AAVALLPAVLLALLAP

SEQ ID NO: 10 - protein, 11 aa, Artificial Sequence
  Membrane translocation sequence-containing peptide RFGF analogue
AALLPVLLAAP

SEQ ID NO: 11 - protein, 13 aa, Artificial Sequence
  HIV Tat protein
GRKKRRQRRRPPQ

SEQ ID NO: 12 - protein, 15 aa, Artificial Sequence
  Drosophila Antennapedia protein
RQIKIWFQNRRMKWK

SEQ ID NO: 13 - protein, 226 aa, Hepatitis B Virus
  HBsAg S domain
MENITSGFLGPLLVLQAGFFLLTRILTIPQSLDSWWTSLNFLGGTTVCLGQNSQSPTSNHSPTSCPPTCPGYRWMCLRRFIIFLFILLLCLIFLLVLLDYQGMLPVCPLIPGSSTTSTGPCRTCMTTAQGTSMYPSCCCTKPSDGNCTCIPIPSSWAFGKFLWEWASARFSWLSLLVPFVQWFVGLSPTVWLSVIWMMWYWGPSLYSILSPFLPLLPIFFCLWVYI

SEQ ID NO: 14 - protein, 72 aa, Hepatitis B Virus
  J02203 (D, ayw3) HBsAg Antigenic Loop Sequence
QGMLPVCPLIPGSSTTSTGPCRTCMTTAQGTSMYPSCCCTKPSDGNCTCIPIPSSWAFGKFLWEWASARFSW

SEQ ID NO: 15 - protein, 72 aa, Hepatitis B Virus
  FJ899792 (D, adw2) HBsAg Antigenic Loop Sequence
QGMLPVCPLIPGSSTTGTGPCRTCTTPAQGTSMYPSCCCTKPSDGNCTCIPIPSSWAFGKFLWEWASARFSW

SEQ ID NO: 16 - protein, 72 aa, Hepatitis B Virus
  AM282986 (A) HBsAg Antigenic Loop Sequence
QGMLPVCPLIPGTTTTSTGPCKTCTTPAQGNSMFPSCCCTKPSDGNCTCIPIPSSWAFAKYLWEWASVRFSW

SEQ ID NO: 17 - protein, 72 aa, Hepatitis B Virus
  D23678 (B1) HBsAg Antigenic Loop Sequence
QGMLPVCPLIPGSSTTSTGPCKTCTTPAQGTSMFPSCCCTKPTDGNCTCIPIPSSWAFAKYLWEWASVRFSW

SEQ ID NO: 18 - protein, 72 aa, Hepatits B Virus
  AB117758 (C1) HBsAg Antigenic Loop Sequence
QGMLPVCPLLPGTSTTSTGPCKTCTIPAQGTSMFPSCCCTKPSDGNCTCIPIPSSWAFARFLWEWASVRFSW

SEQ ID NO: 19 - protein, 74 aa, Hepatitis B Virus
  AB205192(E) HBsAg Antigenic Loop Sequence
QGMLPVCPLIPGSSTTSTGPCRTCTTLAQGTSMFPSCCCSKPSDGNCTCIPIPSSWAFGKFLWEWASARFSWLS

SEQ ID NO: 20 - protein, 71 aa, Hepatitis B Virus
  X69798 (F4) HBsAg Antigenic Loop Sequence
QGMLPVCPLLPGSTTTSTGPCTCTTLAQGTSMFPSCCCSKPSDGNCTCIPIPSSWALGKYLWEWASARFSW

SEQ ID NO: 21 - protein, 70 aa, Hepatitis B Virus
  AF1 60501 (G) HBsAg Antigenic Loop Sequence
QGMLPVCPLIPGSSTTSTGPCTCTTPAQGNSMYPSCCCTPSDGNCTCIPIPSSWAFAKYLWEWASVRFSW

SEQ ID NO: 22 - protein, 72 aa, Hepatitis B Virus
  AY090454 (H) HBsAg Antigenic Loop Sequence
QGMLPVCPLLPGSTTTSTGPCKTCTTLAQGTSMFPSCCCTKPSDGNCTCIPIPSSWAFGKYLWEWASARFSW

SEQ ID NO: 23 - protein, 72 aa, Hepatitis B Virus
  AF241409 (I) HBsAg Antigenic Loop Sequence
QGMLPVCPLIPGSSTTSTGPCKTCTTPAQGNSMYPSCCCTKPSDGNCTCIPIPSSWAFAKYLWEWASARFSW

SEQ ID NO: 24 - protein, 72 aa, Hepatitis B Virus
  AB486012 (J) HBsAg Antigenic Loop Sequence
QGMLPVCPLLPGSTTTSTGPCRTCTITAQGTSMFPSCCCTKPSDGNCTCIPIPSSWAFAKFLWEWASVRFSW

SEQ ID NO: 25 - protein, 72 aa, Hepatitis B Virus
  HBsAg Y100C/P120T HBsAg Antigenic Loop Sequence
CQGMLPVCPLIPGSSTTGTGTCRTCTTPAQGTSMYPSCCCTKPSDGNCTCIPIPSSWAFGFLWEWASARFSW

SEQ ID NO: 26 - protein, 72 aa, Hepatitis B Virus
  HBsAg P120T HBsAg Antigenic Loop Sequence
QGMLPVCPLIPGSSTTGTGTCRTCTTPAQGTSMYPSCCCTKPSDGNCTCIPIPSSWAFGKFLWEWASARFSW

SEQ ID NO: 27 - protein, 72 aa, Hepatitis B Virus
  HBsAg P120T/S143L HBsAg Antigenic Loop Sequence
QGMLPVCPLIPGSSTTGTGTCRTCTTPAQGTSMYPSCCCTKPLDGNCTCIPIPSSWAFGKFLWEWASARFSW

SEQ ID NO: 28 - protein, 72 aa, Hepatitis B Virus
  HBsAg C121 S HBsAg Antigenic Loop Sequence
QGMLPVCPLIPGSSTTGTGPSRTCTTPAQGTSMYPSCCCTKPSDGNCTCIPIPSSWAFGKFLWEWASARFSW

SEQ ID NO: 29 - protein, 72 aa, Hepatitis B Virus
  HBsAg R122D HBsAg Antigenic Loop Sequence
QGMLPVCPLIPGSSTTGTGPCDTCTTPAQGTSMYPSCCCTKPSDGNCTCIPIPSSWAFGKFLWEWASARFSW

SEQ ID NO: 30 - protein, 71 aa, Hepatitis B Virus
  HBsAg R122I HBsAg Antigenic Loop Sequence
QGMLPVCPLIPGSSTTGTGPCITCTTPAQGTSMYPSCCCTPSDGNCTCIPIPSSWAFGKFLWEWASARFSW

SEQ ID NO: 31 - protein, 72 aa, Hepatitis B Virus
  HBsAg T123N HBsAg Antigenic Loop Sequence
QGMLPVCPLIPGSSTTGTGPCRNCTTPAQGTSMYPSCCCTKPSDGNCTCIPIPSSWAFGKFLWEWASARFSW

SEQ ID NO: 32 - protein, 72 aa, Hepatitis B Virus
  HBsAg Q129H HBsAg Antigenic Loop Sequence
QGMLPVCPLIPGSSTTGTGPCRTCTTPAHGTSMYPSCCCTKPSDGNCTCIPIPSSWAFGKFLWEWASARFSW

SEQ ID NO: 33 - protein, 72 aa, Hepatitis B Virus
  HBsAg Q129L HBsAg Antigenic Loop Sequence
QGMLPVCPLIPGSSTTGTGPCRTCTTPALGTSMYPSCCCTKPSDGNCTCIPIPSSWAFGKFLWEWASARFSW

SEQ ID NO: 34 - protein, 72 aa, Hepatitis B Virus
  HBsAg M1 33H HBsAg Antigenic Loop Sequence
QGMLPVCPLIPGSSTTGTGPCRTCTTPAQGTSHYPSCCCTKPSDGNCTCIPIPSSWAFGKFLWEWASARFSW

SEQ ID NO: 35 - protein, 72 aa, Hepatitis B Virus
  HBsAg M1 33L HBsAg Antigenic Loop Sequence
QGMLPVCPLIPGSSTTGTGPCRTCTTPAQGTSLYPSCCCTKPSDGNCTCIPIPSSWAFGKFLWEWASARFSW

SEQ ID NO: 36 - protein, 72 aa, Hepatitis B Virus
  HBsAg M133T HBsAg Antigenic Loop Sequence
QGMLPVCPLIPGSSTTGTGPCRTCTTPAQGTSTYPSCCCTKPSDGNCTCIPIPSSWAFGKFLWEWASARFSW

SEQ ID NO: 37 - protein, 72 aa, Hepatitis B Virus
  HBsAg K141 E HBsAg Antigenic Loop Sequence
QGMLPVCPLIPGSSTTGTGPCRTCTTPAQGTSMYPSCCCTEPSDGNCTCIPIPSSWAFGKFLWEWASARFSW

SEQ ID NO: 38 - protein, 72 aa, Hepatitis B Virus
  HBsAg P142S HBsAg Antigenic Loop Sequence
QGMLPVCPLIPGSSTTGTGPCRTCTTPAQGTSMYPSCCCTKSSDGNCTCIPIPSSWAFGKFLWEWASARFSW

SEQ ID NO: 39 - protein, 72 aa, Hepatitis B Virus
  HBsAg S143K HBsAg Antigenic Loop Sequence
QGMLPVCPLIPGSSTTGTGPCRTCTTPAQGTSMYPSCCCTKPKDGNCTCIPIPSSWAFGKFLWEWASARFSW

SEQ ID NO: 40 - protein, 71 aa, Hepatitis B Virus
  HBsAg D144A HBsAg Antigenic Loop Sequence
QGMLPVCPLIPGSSTTGTGPCRTCTTPAQGTSMYPSCCCTPSAGNCTCIPIPSSWAFGKFLWEWASARFSW

SEQ ID NO: 41 - protein, 72 aa, Hepatitis B Virus
  HBsAg G145R HBsAg Antigenic Loop Sequence
QGMLPVCPLIPGSSTTGTGPCRTCTTPAQGTSMYPSCCCTKPSDRNCTCIPIPSSWAFGKFLWEWASARFSW

SEQ ID NO: 42 - protein, 72 aa, Hepatitis B Virus
  HBsAg N146A HBsAg Antigenic Loop Sequence
QGMLPVCPLIPGSSTTGTGPCRTCTTPAQGTSMYPSCCCTKPSDGACTCIPIPSSWAFGKFLWEWASARFSW

SEQ ID NO: 43 - protein, 226 aa, Hepatitis B Virus
  HBsAg Genotype D S domain (Genbank accession no. FJ899792)
MENVTSGFLGPLLVLQAGFFLLTRILTIPQSLDSWWTSLNFLGGTTVCLGQNSQSPTSNHSPTSCPPTCPGYRWMCLRRFIIFLFILLLCLIFLLVLLDYQGMLPVCPLIPGSSTTGTGPCRTCTTPAQGTSMYPSCCCTKPSDGNCTCIPIPSSWAFGKFLWEWASARFSWLSLLVPFVQWFVGLSPTVWLSVIWMMWYWGPSLYSTLSPFLPLLPIFFCLWVYI

SEQ ID NO: 44 - protein, 8 aa, Artificial Sequence
  Synthetic sequence HBC34 CDRH1
GRIFRSFY

SEQ ID NO: 45 - protein, 7 aa, Artificial Sequence
  Synthetic sequence HBC34 short CDRH2
NQDGSEK

SEQ ID NO: 46 - protein, 8 aa, Artificial Sequence
  Synthetic sequence HBC34 long CDRH2
INQDGSEK

SEQ ID NO: 47 - protein, 12 aa, Artificial Sequence
  Synthetic sequence HBC34 CDRH3
AAWSGNSGGMDV

SEQ ID NO: 48 - protein, 6 aa, Artificial Sequence
  Synthetic sequence HBC34 CDRL1
KLGNKN

SEQ ID NO: 49 - protein, 3 aa, Artificial Sequence
  Synthetic sequence HBC34 short CDRL2
EVK

SEQ ID NO: 50 - protein, 9 aa, Artificial Sequence
  Synthetic sequence HBC34 long CDRL2
VIYEVKYRP

SEQ ID NO: 51 - protein, 9 aa, Artificial Sequence
  Synthetic sequence HBC34 CDRL3
QTWDSTTVV

SEQ ID NO: 52 - protein, 9 aa, Artificial Sequence
  Synthetic sequence HBC34v35 CDRL3
QTFDSTTVV

SEQ ID NO: 53 - protein, 119 aa, Artificial Sequence
  Synthetic sequence HBC34 VH
ELQLVESGGGWVQPGGSQRLSCAASGRIFRSFYMSWVRQAPGKGLEWVATINQDGSEKLYVDSVKGRFTISRDNAKNSLFLQMNNLRVEDTAVYYCAAWSGNSGGMDVWGQGTTVSVSS

SEQ ID NO: 54 - protein, 119 aa, Artificial Sequence
  Synthetic sequence HBC34v31 VH
EVQLVESGGGLVQPGGSLRLSCAASGRIFRSFYMSWVRQAPGKGLEWVANINQDGSEKLYVDSVKGRFTISRDNAKNSLFLQMNNLRVEDTAVYYCAAWSGNSGGMDVWGQGTTVTVSS

SEQ ID NO: 55 - protein, 106 aa, Artificial Sequence
  Synthetic sequence HBC34 VL
SYELTQPPSVSVSPGQTVSIPCSGDKLGNKNVCWFQHKPGQSPVLVIYEVKYRPSGIPERFSGSNSGNTATLTISGTQAMDEAAYFCQTWDSTTVVFGGGTRLTVL

SEQ ID NO: 56 - protein, 106 aa, Artificial Sequence
  Synthetic sequence HBC34v7 VL
SYELTQPPSVSVSPGQTVSIPCSGDKLGNKNVCWFQHKPGQSPVLVIYEVKYRPSGIPERFSGSNSGNTATLTISGTQAMDEAAYFCQTFDSTTVVFGGGTRLTVL

SEQ ID NO: 57 - protein, 106 aa, Artificial Sequence
  Synthetic sequence HBC34v23 VL
SYELTQPPSVSVSPGQTASITCSGDKLGNKNACWYQQKPGQSPVLVIYEVKYRPSGIPERFSGSNSGNTATLTISGTQAMDEADYYCQTFDSTTVVFGGGTKLTVL

SEQ ID NO: 58 - protein, 106 aa, Artificial Sequence
  Synthetic sequence HBC34v34 VL
SYELTQPPSVSVSPGQTVSIPCSGDKLGNKNVSWFQHKPGQSPVLVIYEVKYRPSGIPERFSGSNSGNTATLTISGTQAMDEAAYFCQTFDSTTVVFGGGTRLTVL

SEQ ID NO: 59 - protein, 106 aa, Artificial Sequence
  Synthetic sequence HBC34v35 VL
SYELTQPPSVSVSPGQTVSIPCSGDKLGNKNVAWFQHKPGQSPVLVIYEVKYRPSGIPERFSGSNSGNTATLTISGTQAMDEAAYFCQTFDSTTVVFGGGTRLTVL

SEQ ID NO: 60 - protein, 106 aa, Artificial Sequence
  Synthetic sequence HBC34_LC40S VL
SYELTQPPSVSVSPGQTVSIPCSGDKLGNKNVSWFQHKPGQSPVLVIYEVKYRPSGIPERFSGSNSGNTATLTISGTQAMDEAAYFCQTWDSTTVVFGGGTRLTVL

SEQ ID NO: 61 - protein, 106 aa, Artificial Sequence
  Synthetic sequence HBC34_LC40A VL
SYELTQPPSVSVSPGQTVSIPCSGDKLGNKNVAWFQHKPGQSPVLVIYEVKYRPSGIPERFSGSNSGNTATLTISGTQAMDEAAYFCQTWDSTTVVFGGGTRLTVL

SEQ ID NO: 62 - protein, 106 aa, Artificial Sequence
  Synthetic sequence HBC34v23_LC40S VL
SYELTQPPSVSVSPGQTASITCSGDKLGNKNASWYQQKPGQSPVLVIYEVKYRPSGIPERFSGSNSGNTATLTISGTQAMDEADYYCQTFDSTTVVFGGGTKLTVL

SEQ ID NO: 63 - protein, 106 aa, Artificial Sequence
  Synthetic sequence HBC34v23_LC40A VL
SYELTQPPSVSVSPGQTASITCSGDKLGNKNAAWYQQKPGQSPVLVIYEVKYRPSGIPERFSGSNSGNTATLTISGTQAMDEADYYCQTFDSTTVVFGGGTKLTVL

SEQ ID NO: 64 - protein, 106 aa, Artificial Sequence; identical to SEQ ID NO: 60
  Synthetic sequence HBC34v31_LC40S VL

SEQ ID NO: 65 - protein, 106 aa, Artificial Sequence; identical to SEQ ID NO: 61
  Synthetic sequence HBC34v31_L C40A VL

SEQ ID NO: 66 - protein, 106 aa, Artificial Sequence; identical to SEQ ID NO: 58
  Synthetic sequence HBC34v32_LC40S VL

SEQ ID NO: 67 - protein, 106 aa, Artificial Sequence; identical to SEQ ID NO: 59
  Synthetic sequence HBC34v32_LC40A VL

SEQ ID NO: 68 - protein, 106 aa, Artificial Sequence; identical to SEQ ID NO: 62
  Synthetic sequence HBC34v33_LC40S VL

SEQ ID NO: 69 - protein, 106 aa, Artificial Sequence; identical to SEQ ID NO: 63
  Synthetic sequence HBC34v33_LC40A VL

SEQ ID NO: 70 - protein, 449 aa, Artificial Sequence
  Synthetic sequence HBC34v35 HC
ELQLVESGGGWVQPGGSQRLSCAASGRIFRSFYMSWVRQAPGKGLEWVATINQDGSEKLYVDSVKGRFTISRDNAKNSLFLQMNNLRVEDTAVYYCAAWSGNSGGMDVWGQGTTVSVSSASTKGPSVFPLAPSSKSTSGGTAALGCLVKDYFPEPVTVSWNSGALTSGVHTFPAVLQSSGLYSLSSVVTVPSSSLGTQTYICNVNHKPSNTKVDKKVEPKSCDKTHTCPPCPAPELLGGPSVFLFPPKPKDTLMISRTPEVTCVVVDVSHEDPEVKFNWYVDGVEVHNAKTKPREEQYNSTYRVVSVLTVLHQDWLNGKEYKCKVSNKALPAPIEKTISKAKGQPREPQVYTLPPSRDELTKNQVSLTCLVKGFYPSDIAVEWESNGQPENNYKTTPPVLDSDGSFFLYSKLTVDKSRWQQGNVFSCSVMHEALHNHYTQKSLSLSPGK

SEQ ID NO: 71 - protein, 449 aa, Artificial Sequence
  Synthetic sequence HBC34v35-MLNS-GAALIE (g1M17, 1) HC
ELQLVESGGGWVQPGGSQRLSCAASGRIFRSFYMSWVRQAPGKGLEWVATINQDGSEKLYVDSVKGRFTISRDNAKNSLFLQMNNLRVEDTAVYYCAAWSGNSGGMDVWGQGTTVSVSSASTKGPSVFPLAPSSKSTSGGTAALGCLVKDYFPEPVTVSWNSGALTSGVHTFPAVLQSSGLYSLSSVVTVPSSSLGTQTYICNVNHKPSNTKVDKKVEPKSCDKTHTCPPCPAPELLAGPSVFLFPPKPKDTLMISRTPEVTCVVVDVSHEDPEVKFNWYVDGVEVHNAKTKPREEQYNSTYRVVSVLTVLHQDWLNGKEYKCKVSNKALPLPEEKTISKAKGQPREPQVYTLPPSRDELTKNQVSLTCLVKGFYPSDIAVEWESNGQPENNYKTTPPVLDSDGSFFLYSKLTVDKSRWQQGNVFSCSVLHEALHSHYTQKSLSLSPGK

SEQ ID NO: 72 - protein, 449 aa, Artificial Sequence
  Synthetic sequence HBC34v35-MLNS HC
ELQLVESGGGWVQPGGSQRLSCAASGRIFRSFYMSWVRQAPGKGLEWVATINQDGSEKLYVDSVKGRFTISRDNAKNSLFLQMNNLRVEDTAVYYCAAWSGNSGGMDVWGQGTTVSVSSASTKGPSVFPLAPSSKSTSGGTAALGCLVKDYFPEPVTVSWNSGALTSGVHTFPAVLQSSGLYSLSSVVTVPSSSLGTQTYICNVNHKPSNTKVDKKVEPKSCDKTHTCPPCPAPELLGGPSVFLFPPKPKDTLMISRTPEVTCVVVDVSHEDPEVKFNWYVDGVEVHNAKTKPREEQYNSTYRVVSVLTVLHQDWLNGKEYKCKVSNKALPAPIEKTISKAKGQPREPQVYTLPPSRDELTKNQVSLTCLVKGFYPSDIAVEWESNGQPENNYKTTPPVLDSDGSFFLYSKLTVDKSRWQQGNVFSCSVLHEALHSHYTQKSLSLSPGK

SEQ ID NO: 73 - protein, 212 aa, Artificial Sequence
  Synthetic sequence HBC34v35 LC
SYELTQPPSVSVSPGQTVSIPCSGDKLGNKNVAWFQHKPGQSPVLVIYEVKYRPSGIPERFSGSNSGNTATLTISGTQAMDEAAYFCQTFDSTTVVFGGGTRLTVLGQPKAAPSVTLFPPSSEELQANKATLVCLISDFYPGAVTVAWKADSSPVKAGVETTTPSKQSNNKYAASSYLSLTPEQWKSHRSYSCQVTHEGSTVEKTVAPTECS

SEQ ID NO: 74 - protein, 212 aa, Artificial Sequence
  Synthetic sequence HBC34v34 LC
SYELTQPPSVSVSPGQTVSIPCSGDKLGNKNVSWFQHKPGQSPVLVIYEVKYRPSGIPERFSGSNSGNTATLTISGTQAMDEAAYFCQTFDSTTVVFGGGTRLTVLGQPKAAPSVTLFPPSSEELQANKATLVCLISDFYPGAVTVAWKADSSPVKAGVETTTPSKQSNNKYAASSYLSLTPEQWKSHRSYSCQVTHEGSTVEKTVAPTECS

SEQ ID NO: 75 - protein, 128 aa, Artificial Sequence
  Synthetic sequence HBC24 VH
EVQLLESGGGLVQPGGSLRLSCAASGSTFTKYAMSWVRQAPGKGLEWVASISGSVPGFGIDTYYADSVKGRFTISRDTSKNTLYLQMNSLRAEDTALYYCAKDVGVIGSYYYYAMDVWGQGTAVTVSS

SEQ ID NO: 76 - protein, 109 aa, Artificial Sequence
  Synthetic sequence HBC24 VL
EIVLTQSPGTLSLSPGERATLSCRASQGLSSSYLAWYQQKPGQAPRLLIYSASTRATGIPDRFSGSGSGTDFTLTISRLEPEDFAVYYCQQYAYSPRWTFGQGTKVEIK

SEQ ID NO: 77 - protein, 8 aa, Artificial Sequence
  Synthetic sequence HBC24 CDRH1
GSTFTKYA

SEQ ID NO: 78 - protein, 8 aa, Artificial Sequence
  Synthetic sequence HBC24 CDRH2
ISGSVPGF

SEQ ID NO: 79 - protein, 21 aa, Artificial Sequence
  Synthetic sequence HBC24 CDRH3
LYYCAKDVGVIGSYYYYAMDV

SEQ ID NO: 80 - protein, 7 aa, Artificial Sequence
  Synthetic sequence HBC24 CDRL1
QGLSSSY

SEQ ID NO: 81 - protein, 3 aa, Artificial Sequence
  Synthetic sequence HBC24 CDRL2
SAS

SEQ ID NO: 82 - protein, 10 aa, Artificial Sequence
  Synthetic sequence HBC24 CDRL3
QQYAYSPRWT

SEQ ID NO: 83 - protein, 212 aa, Artificial Sequence
  Synthetic sequence HBC34 LC
SYELTQPPSVSVSPGQTVSIPCSGDKLGNKNVCWFQHKPGQSPVLVIYEVKYRPSGIPERFSGSNSGNTATLTISGTQAMDEAAYFCQTWDSTTVVFGGGTRLTVLGQPKAAPSVTLFPPSSEELQANKATLVCLISDFYPGAVTVAWKADSSPVKAGVETTTPSKQSNNKYAASSYLSLTPEQWKSHRSYSCQVTHEGSTVEKTVAPTECS

SEQ ID NO: 84 - protein, 212 aa, Artificial Sequence
  Synthetic sequence HBC34v7 LC
SYELTQPPSVSVSPGQTVSIPCSGDKLGNKNVCWFQHKPGQSPVLVIYEVKYRPSGIPERFSGSNSGNTATLTISGTQAMDEAAYFCQTFDSTTVVFGGGTRLTVLGQPKAAPSVTLFPPSSEELQANKATLVCLISDFYPGAVTVAWKADSSPVKAGVETTTPSKQSNNKYAASSYLSLTPEQWKSHRSYSCQVTHEGSTVEKTVAPTECS

SEQ ID NO: 85 - protein, 212 aa, Artificial Sequence
  Synthetic sequence HBC34v23 LC
SYELTQPPSVSVSPGQTASITCSGDKLGNKNACWYQQKPGQSPVLVIYEVKYRPSGIPERFSGSNSGNTATLTISGTQAMDEADYYCQTFDSTTVVFGGGTKLTVLGQPKAAPSVTLFPPSSEELQANKATLVCLISDFYPGAVTVAWKADSSPVKAGVETTTPSKQSNNKYAASSYLSLTPEQWKSHRSYSCQVTHEGSTVEKTVAPTECS

SEQ ID NO: 86 - protein, 212 aa, Artificial Sequence
  Synthetic sequence HBC34_LC40S LC
SYELTQPPSVSVSPGQTVSIPCSGDKLGNKNVSWFQHKPGQSPVLVIYEVKYRPSGIPERFSGSNSGNTATLTISGTQAMDEAAYFCQTWDSTTVVFGGGTRLTVLGQPKAAPSVTLFPPSSEELQANKATLVCLISDFYPGAVTVAWKADSSPVKAGVETTTPSKQSNNKYAASSYLSLTPEQWKSHRSYSCQVTHEGSTVEKTVAPTECS

SEQ ID NO: 87 - protein, 212 aa, Artificial Sequence
  Synthetic sequence HBC34_LC40A LC
SYELTQPPSVSVSPGQTVSIPCSGDKLGNKNVAWFQHKPGQSPVLVIYEVKYRPSGIPERFSGSNSGNTATLTISGTQAMDEAAYFCQTWDSTTVVFGGGTRLTVLGQPKAAPSVTLFPPSSEELQANKATLVCLISDFYPGAVTVAWKADSSPVKAGVETTTPSKQSNNKYAASSYLSLTPEQWKSHRSYSCQVTHEGSTVEKTVAPTECS

SEQ ID NO: 88 - protein, 212 aa, Artificial Sequence
  Synthetic sequence HBC34v23_LC40S LC
SYELTQPPSVSVSPGQTASITCSGDKLGNKNASWYQQKPGQSPVLVIYEVKYRPSGIPERFSGSNSGNTATLTISGTQAMDEADYYCQTFDSTTVVFGGGTKLTVLGQPKAAPSVTLFPPSSEELQANKATLVCLISDFYPGAVTVAWKADSSPVKAGVETTTPSKQSNNKYAASSYLSLTPEQWKSHRSYSCQVTHEGSTVEKTVAPTECS

SEQ ID NO: 89 - protein, 212 aa, Artificial Sequence
  Synthetic sequence HBC34v23_LC40A LC
SYELTQPPSVSVSPGQTASITCSGDKLGNKNAAWYQQKPGQSPVLVIYEVKYRPSGIPERFSGSNSGNTATLTISGTQAMDEADYYCQTFDSTTVVFGGGTKLTVLGQPKAAPSVTLFPPSSEELQANKATLVCLISDFYPGAVTVAWKADSSPVKAGVETTTPSKQSNNKYAASSYLSLTPEQWKSHRSYSCQVTHEGSTVEKTVAPTECS

SEQ ID NO: 90 - protein, 212 aa, Artificial Sequence; identical to SEQ ID NO: 86
  Synthetic sequence HBC34v31_LC40S

SEQ ID NO: 91 - protein, 212 aa, Artificial Sequence; identical to SEQ ID NO: 87
  Synthetic sequence HBC34v31_LC40A LC

SEQ ID NO: 92 - protein, 212 aa, Artificial Sequence; identical to SEQ ID NO: 74
  Synthetic sequence HBC34v32_LC40S LC

SEQ ID NO: 93 - protein, 212 aa, Artificial Sequence; identical to SEQ ID NO: 73
  Synthetic sequence HBC34v32_LC40A LC

SEQ ID NO: 94 - protein, 212 aa, Artificial Sequence; identical to SEQ ID NO: 88
  Synthetic sequence HBC34v33_LC40S LC

SEQ ID NO: 95 - protein, 212 aa, Artificial Sequence; identical to SEQ ID NO: 89
  Synthetic sequence HBC34v33 _LC40A LC

SEQ ID NO: 96 - protein, 217 aa, Homo sapiens
  WT hIgG1 Fc
APELLGGPSVFLFPPKPKDTLMISRTPEVTCVVVDVSHEDPEVKFNWYVDGVEVHNAKTKPREEQYNSTYRVVSVLTVLHQDWLNGKEYKCKVSNKALPAPIEKTISKAKGQPREPQVYTLPPSRDELTKNQVSLTCLVKGFYPSDIAVEWESNGQPENNYKTTPPVLDSDGSFFLYSKLTVDKSRWQQGNVFSCSVMHEALHNHYTQKSLSLSPGK

SEQ ID NO: 97 - protein, 449 aa, Artificial Sequence
  Synthetic sequence HBC34+GAALIE HC
ELQLVESGGGWVQPGGSQRLSCAASGRIFRSFYMSWVRQAPGKGLEWVATINQDGSEKLYVDSVKGRFTISRDNAKNSLFLQMNNLRVEDTAVYYCAAWSGNSGGMDVWGQGTTVSVSSASTKGPSVFPLAPSSKSTSGGTAALGCLVKDYFPEPVTVSWNSGALTSGVHTFPAVLQSSGLYSLSSVVTVPSSSLGTQTYICNVNHKPSNTKVDKKVEPKSCDKTHTCPPCPAPELLAGPSVFLFPPKPKDTLMISRTPEVTCVVVDVSHEDPEVKFNWYVDGVEVHNAKTKPREEQYNSTYRVVSVLTVLHQDWLNGKEYKCKVSNKALPLPEEKTISKAKGQPREPQVYTLPPSRDELTKNQVSLTCLVKGFYPSDIAVEWESNGQPENNYKTTPPVLDSDGSFFLYSKLTVDKSRWQQGNVFSCSVMHEALHNHYTQKSLSLSPGK

SEQ ID NO: 98 - protein, 449 aa, Artificial Sequence
  Synthetic sequence HBC34v31+GAALIE HC
EVQLVESGGGLVQPGGSLRLSCAASGRIFRSFYMSWVRQAPGKGLEWVANINQDGSEKLYVDSVKGRFTISRDNAKNSLFLQMNNLRVEDTAVYYCAAWSGNSGGMDVWGQGTTVTVSSASTKGPSVFPLAPSSKSTSGGTAALGCLVKDYFPEPVTVSWNSGALTSGVHTFPAVLQSSGLYSLSSVVTVPSSSLGTQTYICNVNHKPSNTKVDKKVEPKSCDKTHTCPPCPAPELLAGPSVFLFPPKPKDTLMISRTPEVTCVVVDVSHEDPEVKFNWYVDGVEVHNAKTKPREEQYNSTYRVVSVLTVLHQDWLNGKEYKCKVSNKALPLPEEKTISKAKGQPREPQVYTLPPSRDELTKNQVSLTCLVKGFYPSDIAVEWESNGQPENNYKTTPPVLDSDGSFFLYSKLTVDKSRWQQGNVFSCSVMHEALHNHYTQKSLSLSPGK

SEQ ID NO: 99 - protein, 449 aa, Artificial Sequence
  Synthetic sequence murinized HBC34v7, BC34-v7-mu-IgG2a - HC
ELQLVESGGGWVQPGGSQRLSCAASGRIFRSFYMSWVRQAPGKGLEWVATINQDGSEKLYVDSVKGRFTISRDNAKNSLFLQMNNLRVEDTAVYYCAAWSGNSGGMDVWGQGTTVSVSSAKTTAPSVYPLAPVCGDTTGSSVTLGCLVKGYFPEPVTLTWNSGSLSSGVHTFPAVLQSDLYTLSSSVTVTSSTWPSQSITCNVAHPASSTKVDKKIEPRGPTIKPCPPCKCPAPNLLGGPSVFIFPPKIKDVLMISLSPIVTCVVVDVSEDDPDVQISWFVNNVEVHTAQTQTHREDYNSTLRVVSALPIQHQDWMSGKEFKCKVNNKDLPAPIERTISKPKGSVRAPQVYVLPPPEEEMTKKQVTLTCMVTDFMPEDIYVEWTNNGKTELNYKNTEPVLDSDGSYFMYSKLRVEKKNWVERNSYSCSVVHEGLHNHHTTKSFSRTPGK

SEQ ID NO: 100 - protein, 212 aa, Artificial Sequence
  Synthetic sequence murinized HBC34v7, BC34-v7-mu-IgG2a - LC
SYELTQPPSVSVSPGQTVSIPCSGDKLGNKNVCWFQHKPGQSPVLVIYEVKYRPSGIPERFSGSNSGNTATLTISGTQAMDEAAYFCQTFDSTTVVFGGGTRLTVLGQPKSSPSVTLFPPSSEELETNKATLVCTITDFYPGVVTVDWKVDGTPVTQGMETTQPSKQSNNKYMASSYLTLTARAWERHSSYSCQVTHEGHTVEKSLSRADCS

SEQ ID NO: 101 - protein, 449 aa, Artificial Sequence; identical to SEQ ID NO: 99
  Synthetic sequence murinized HBC34v35, HBC34-v35-mu-IgG2a - HC

SEQ ID NO: 102 - protein, 212 aa, Artificial Sequence
  Synthetic sequence murinized HBC34v35, HBC34-v35-mu-IgG2a - LC
SYELTQPPSVSVSPGQTVSIPCSGDKLGNKNVAWFQHKPGQSPVLVIYEVKYRPSGIPERFSGSNSGNTATLTISGTQAMDEAAYFCQTFDSTTVVFGGGTRLTVLGQPKSSPSVTLFPPSSEELETNKATLVCTITDFYPGVVTVDWKVDGTPVTQGMETTQPSKQSNNKYMASSYLTLTARAWERHSSYSCQVTHEGHTVEKSLSRADCS

SEQ ID NO: 103 - protein, 458 aa, Artificial Sequence
  Synthetic sequence murinized HBC24, HBC24-mu-IgG2a - HC
EVQLLESGGGLVQPGGSLRLSCAASGSTFTKYAMSWVRQAPGKGLEWVASISGSVPGFGIDTYYADSVKGRFTISRDTSKNTLYLQMNSLRAEDTALYYCAKDVGVIGSYYYYAMDVWGQGTAVTVSSAKTTAPSVYPLAPVCGDTTGSSVTLGCLVKGYFPEPVTLTWNSGSLSSGVHTFPAVLQSDLYTLSSSVTVTSSTWPSQSITCNVAHPASSTKVDKKIEPRGPTIKPCPPCKCPAPNLLGGPSVFIFPPKIKDVLMISLSPIVTCVVVDVSEDDPDVQISWFVNNVEVHTAQTQTHREDYNSTLRVVSALPIQHQDWMSGKEFKCKVNNKDLPAPIERTISKPKGSVRAPQVYVLPPPEEEMTKKQVTLTCMVTDFMPEDIYVEWTNNGKTELNYKNTEPVLDSDGSYFMYSKLRVEKKNWVERNSYSCSVVHEGLHNHHTTKSFSRTPGK

SEQ ID NO: 104 - protein, 215 aa, Artificial Sequence
  Synthetic sequence murinized HBC24, HBC24-mu-IgG2a - LC
EIVLTQSPGTLSLSPGERATLSCRASQGLSSSYLAWYQQKPGQAPRLLIYSASTRATGIPDRFSGSGSGTDFTLTISRLEPEDFAVYYCQQYAYSPRWTFGQGTKVEIKADAAPTVSIFPPSSEQLTSGGASVVCFLNNFYPKDINVKWKIDGSERQNGVLNSWTDQDSKDSTYSMSSTLTLTKDEYERHNSYTCEATHKTSTSPIVKSFNRNEC

SEQ ID NO: 105 - protein, 19 aa, Artificial Sequence
  Synthetic sequence chimeric hinge
ESKYGPPCPPCPAPPVAGP

SEQ ID NO: 106 - RNA, 21 nt, Artificial Sequence
  Synthetic sequence siRNA3 sense strand
gguggacuucucucaauuuua

SEQ ID NO: 107 - RNA, 23 nt, Artificial Sequence
  Synthetic sequence siRNA3 antisense strand
uaaaauugagagaaguccaccac

SEQ ID NO: 108 - RNA, 21 nt, Artificial Sequence
  Synthetic oligonucleotide (siRNA3 sense strand)
gguggacuucucucaauuuua

SEQ ID NO: 109 - RNA, 23 nt, Artificial Sequence
  Synthetic oligonucleotide (siRNA3 antisense strand)
uaaaauugagagaaguccaccac